European Patent Application EP 4 649 958 A1, published November 19, 2025. Title: 用于预防猫鼻气管炎、猫杯状病毒病、猫泛白细胞减少症的三联mRNA疫苗及其制备方法. Applicant: 浙江大学. The sequence listing filed with the application follows.

SEQUENCE LISTING (20 sequences)

SEQ ID NO: 1 - DNA, 2508 bp, synthetic construct
  source 1..2508: mol_type = other DNA
atgacaagactgcacttctggtggtgcggcatcttcgccgtgctgaagtacctggtgtgcacaagcagcagcacccggggcgacctgggcaagagacggagaggcagcagatggcaaggccacagcggctacttcagacagagatgcttcttccctagcctgctgggcatcgccgccaccggcagcagacacggcaacggcagcagcggcctgacaagactggctagatacgtgagcttcatctggatcgtgctgttcctggtgggccctagacccgtggaggggcagagcggcagcacaagcgaacagcctagaagaaccgtggccacccccgaggtcggcggcaccccccccaagcccaccaccgaccccaccgacatgtccgacatgagagaggccctgagagctagccaaatcgaggccaacggccctagcaccttctacatgtgcccccctccctccggcagcaccgtggtgagactggagccccctagagcctgccccgactacaagctgggcaagaacttcaccgagggcatcgccgtgatcttcaaggagaacatcgccccctacaagttcaaggccaacatctactacaagaacatcatcatgaccaccgtgtggagcggcagcagctacgccgtgaccaccaacagatacaccgacagagtgcccgtgaaggtgcaagagatcaccgacctgatcgacagaagaggcatgtgcctgagcaaggccgattacgtgagaaacaactatcagttcaccgccttcgacagagacgaggaccctagagagctgcccctgaagcctagcaagttcaacacccccgagagcagaggctggcacaccaccaacgaaacctacaccaagatcggcgccgccggcttccaccacagcggcacaagcgtgaactgcatcgtggaagaggtggacgctagaagcgtgtacccctacgacagcttcgccatctccaccggcgacgtgattcacatgagccccttcttcggcctgagagacggcgcccacgtggagcacacaagctacagcagcgacagatttcagcagatcgagggctactaccccatcgacctggacacaagactgcagctgggcgcccccgtgagcagaaacttcctggaaaccccccacgtgaccgtggcctggaactggacccccaagagcggcagagtgtgcaccctggccaagtggagagagatcgacgaaatgctgagagacgagtaccaaggcagctacagattcaccgccaagaccatcagcgccaccttcatcagcaacacaagccaattcgagatcaacagaatcagactgggcgactgcgccaccaaggaggccgccgaggccatcgacagaatctacaagagcaagtacagcaagacccacattcagaccggcaccctggaaacctacctggctagaggcggcttcctgatcgccttcagacccatgatcagcaatgagctggccaagctgtacatcaacgagctggctagaagcaacagaaccgtggacctgagcgccctgctgaaccctagcggcgaaaccgtgcagagaacaagaagaagcgtgcctagcaatcagcaccacagaagcagaagaagcaccatcgagggcggcatcgaaaccgtgaacaatgcttccctgctgaagaccacaagcagcgtggagttcgccatgctgcagttcgcctacgactacatccaagcccacgtgaacgagatgctgagcagaatcgccaccgcctggtgcaccctgcagaacagagagcacgtgctgtggaccgaaaccctgaagctgaaccccggcggcgtggtgagcatggccctggagagaagagtgagcgctagactgctgggcgacgccgtggccgtgacacagtgcgtgaacatcagcagcggccacgtgtacattcagaacagcatgagagtgaccggcagcagcaccacctgctacagcagacccctggtgagcttcagagccctgaacgacagcgagtacatcgaggggcagctgggcgagaacaacgagctgctggtggagagaaagctgatcgagccctgcaccgtgaacaacaagagatacttcaagttcggcgctgactacgtgtacttcgaggactacgcctacgtgagaaaagtgcccctgagcgagatcgagctgatcagcgcctacgtggacctgaacctgaccctgctggaggacagagagttcctgcccctggaggtgtacacaagagccgagctggaggacaccggcctgctggactacagcgagattcagagaagaaatcagctgcacgccctgaagttctacgacatcgacagcatcgtgagagtggacaacaacctggtgatcatgagagggatggccaactttttccaaggcctcggcgacgtcggcgctggcttcggcaaagtggtgctgggcgccgcctccgccgtgatcagcaccgtgagcggcgtgagcagcttcctgaacaaccccttctag

SEQ ID NO: 2 - DNA, 990 bp, synthetic construct
  source 1..990: mol_type = other DNA
atgatgacaagactgcacttctggtggtgcggcatcttcgccgtgctgaagtacctggtgtgcacaagcagcctgaccacaacccccaagaccacaaccgtgtacgtgaagggcttcaacatcccccccctgagatacaactacacccaagctagaatcgtgcccaagatcccccaagccatggaccccaagatcaccgccgaggtgagatacgtgacaagcatggacagctgcggcatggtggccctgatcagcgagcccgacatcgacgctaccatcagaacaattcagctgagccaaaagaagacctacaatgctaccatcagctggttcaaggtgacccaaggctgcgagtaccccatgttcctgatggacatgagactgtgcgaccccaagagagagttcggcatctgcgccctgagaagccctagctactggctggagcccctgaccaagtacatgttcctgaccgacgacgagctgggcctgatcatgatggcccccgctcagttcaaccaagggcagtacagaagagtgatcaccatcgacggcagcatgttctacaccgacttcatggtgcagctgagccccaccccctgctggttcgccaagcccgacagatacgaggagatcctgcacgagtggtgcagaaacgtgaagaccatcggcctggacggcgctagagactaccactactactgggtgccctacaaccctcagccccaccacaaggccgtgctgctgtactggtacagaacccacggcagagagccccccgtgagattccaagaggccatcagatacgacagacccgccatccctagcggcagcgaggacagcaagagaagcaacgacagcagaggcgagagcagcggccccaactggatcgacatcgagaactacacccccaagaacaacgtgcccatcattatcagcgacgatgacgtgcccaccgccccccccaagggcatgaacaatcagagcgtgtag

SEQ ID NO: 3 - DNA, 1716 bp, synthetic construct
  source 1..1716: mol_type = other DNA
atgggcacaagactgcacttctggtggtgcggcatcttcgccgtgctgaagtacctcgtgtgcacaagcagcgccgacgacggcagcattacagcccccgagcaaggcacaatggtgggcggcgtgattgccgagcctagcgctcagatgagcaccgccgccgacatggccaccggcaagagcgtggacagcgagtgggaggccttcttcagcttccacacaagcgtgaactggagcacaagcgaaacccaaggcaagatcctgttcaagcagagcctgggccccctgctgaacccctacctggagcacctggccaagctgtacgtggcctggagcggcagcatcgaggtgagattcagcattagcggcagcggggtgttcggcggcaaactcgccgccatcgtggtgcctcctggcgtggaccccgtgcagagcacaagcatgctgcagtacccccacgtgctgttcgacgctagacaagtggagcccgtgatcttcagcatccccgacctgagaagcaccctgtaccacctgatgagcgacacagacaccacaagcctggtgatcatggtgtacaacgacctgatcaacccctacgccaacgacgccaacagcagcggctgcatcgtgaccgtggaaaccaagcccggccccgacttcaagttccacctgctgaagccccccggcagcatgctgacccacggcagcgtgcctagcgacctgatccccaagacaagcagcctgtggatcggcaacagatactggagcgacatcaccgacttcgtgatcagacccttcgtgttccaagccaacagacacttcgacttcaaccaagaaaccgccggctggagcacccctagattcagacccatcagcgtgaccatcagcgagcagaacggcgccaagctgggcatcggcgtggccaccgactacatcgtccccgggatccctgacggctggcccgacaccaccatccccggcgaactgatccccgccggcgactacgccatcaccaacggcaccggcaacgacattaccaccgctaccggctacgacaccgccgacatcatcaagaacaacaccaacttcagaggcatgtacatctgcggcagcctgcagagagcctggggcgacaagaagatcagcaacaccgccttcatcaccacagccaccctggacggcgacaacaataacaagatcaacccctgcaacaccatcgatcagagcaagatcgtggtgttccaagacaaccacgtgggcaagaaggtgcagatcagcgacgacaccctggccctgctgggctacaccggcatcggcgagcaagccatcggcagcgacagagacagagtggtgagaatcagcaccctgcccgaaaccggcgctagaggcggcaaccaccccatcttctacaagaacagcatcaagctgggctacgtgatcagaagcatcgacgtgttcaacagccaaatcctgcacacaagcagacagctgagcctgaaccactacctgctgcccctggacagcttcgccgtgtacagaatcatcgacagcggcggcagctggttcgacatcggcatcgattccgacggcttcagcttcgtgggcgtgagcggcttcggcaagctggagttccccctgagcgctagctacatgggcattcagctggccaagatcagactggctagcaacatcagaagccccatgaccaagctgtag

SEQ ID NO: 4 - DNA, 1821 bp, synthetic construct
  source 1..1821: mol_type = other DNA
atgacaagactgcacttctggtggtgcggcatcttcgccgtgctgaagtatctggtctgcacaagcagcagcgacggcgccgtgcagcccgacggcgggcagcctgccgtgagaaacgagcgggctaccggcagcgggaacgggtccggcgggggcggcggggggggcagcggcggcgtgggcatcagcaccggcacatttaacaatcagaccgagttcaagttcctggagaacggctgggtggagatcaccgccaacagcagcagactggtgcacctgaacatgcccgagagcgagaactacaagagagtggtcgtgaacaacatggacaagaccgccgtgaagggcaacatggccctggacgacacccacgtgcagatcgtgaccccctggagcctggtggacgccaacgcctggggcgtgtggttcaaccccggcgactggcagctgatcgtgaacaccatgagcgagctgcacctggtgagcttcgagcaagagatcttcaacgtggtgctgaagaccgtgagcgagagcgccacacagccccccaccaaggtgtacaacaacgacctgaccgctagcctgatggtggccctggacagcaacaacaccatgcccttcacccccgccgccatgagaagcgaaaccctgggcttctacccctggaagcccaccatccccaccccctggagatactactttcagtgggacagaaccctgatccctagccacaccggcacaagcggcacccccaccaacgtgtactacggcaccgaccccgacgacgtgcagttctacaccatcgagaacagcgtgcccgtgcacctgctgagaaccggcgacgagttcgccaccggcaccttttttttcgactgcaagccctgcagactgacccacacctggcagaccaacagagccctgggcctgccccccttcctgaacagcctgcctcagagcgagggcgccaccaacttcggcgacatcggcgtgcagcaagacaagagaagaggcgtgacacagatgggcaacaccgactacatcaccgaggccaccatcatgcggcccgccgaggtgggctacagcgccccctactacagcttcgaggctagcacccaaggccccttcaagacacccatcgccgccggcagaggcggggctcagaccgacgagaaccaagccgccgacggcgaccctagatacgccttcggcagacagcacgggcagaagaccacaaccaccggcgaaacccccgagagactgacctacatcgcccaccaagacaccggcagataccccgagggcgactggattcagaacatcaacttcaacctgcccgtgaccaacgacaacgtgctgctgcccaccgaccccatcggcggcaagaccggcatcaactacaccaacatcttcaacacctacggccccctgaccgccctgaacaacgtgccccccgtgtaccccaacgggcagatctgggacaaggagttcgacaccgacctgaagcctagactgcacgtgaacgcccccttcgtgtgtcagaacaactgccccgggcagctgttcgtgaaggtggcccccaacctgaccaacgagtacgaccccgacgctagcgccaacatgagcagaatcgtgacctacagcgacttctggtggaagggcaagctggtgttcaaggccaagctgagagctagccacacctggaaccccattcagcagatgagcatcaacgtggacaatcagttcaactacgtgcccaacaacatcggcgccatgaagatcgtgtacgagaagagccaactggcccctagaaagctgtactga

SEQ ID NO: 5 - RNA, 2704 nt, synthetic construct
  source 1..2704: mol_type = other RNA
gggaaataagagagaaaagaagagtaagaagaaatataagaccccggcgccgccaccatgacaagactgcacttctggtggtgcggcatcttcgccgtgctgaagtacctggtgtgcacaagcagcagcacccggggcgacctgggcaagagacggagaggcagcagatggcaaggccacagcggctacttcagacagagatgcttcttccctagcctgctgggcatcgccgccaccggcagcagacacggcaacggcagcagcggcctgacaagactggctagatacgtgagcttcatctggatcgtgctgttcctggtgggccctagacccgtggaggggcagagcggcagcacaagcgaacagcctagaagaaccgtggccacccccgaggtcggcggcaccccccccaagcccaccaccgaccccaccgacatgtccgacatgagagaggccctgagagctagccaaatcgaggccaacggccctagcaccttctacatgtgcccccctccctccggcagcaccgtggtgagactggagccccctagagcctgccccgactacaagctgggcaagaacttcaccgagggcatcgccgtgatcttcaaggagaacatcgccccctacaagttcaaggccaacatctactacaagaacatcatcatgaccaccgtgtggagcggcagcagctacgccgtgaccaccaacagatacaccgacagagtgcccgtgaaggtgcaagagatcaccgacctgatcgacagaagaggcatgtgcctgagcaaggccgattacgtgagaaacaactatcagttcaccgccttcgacagagacgaggaccctagagagctgcccctgaagcctagcaagttcaacacccccgagagcagaggctggcacaccaccaacgaaacctacaccaagatcggcgccgccggcttccaccacagcggcacaagcgtgaactgcatcgtggaagaggtggacgctagaagcgtgtacccctacgacagcttcgccatctccaccggcgacgtgattcacatgagccccttcttcggcctgagagacggcgcccacgtggagcacacaagctacagcagcgacagatttcagcagatcgagggctactaccccatcgacctggacacaagactgcagctgggcgcccccgtgagcagaaacttcctggaaaccccccacgtgaccgtggcctggaactggacccccaagagcggcagagtgtgcaccctggccaagtggagagagatcgacgaaatgctgagagacgagtaccaaggcagctacagattcaccgccaagaccatcagcgccaccttcatcagcaacacaagccaattcgagatcaacagaatcagactgggcgactgcgccaccaaggaggccgccgaggccatcgacagaatctacaagagcaagtacagcaagacccacattcagaccggcaccctggaaacctacctggctagaggcggcttcctgatcgccttcagacccatgatcagcaatgagctggccaagctgtacatcaacgagctggctagaagcaacagaaccgtggacctgagcgccctgctgaaccctagcggcgaaaccgtgcagagaacaagaagaagcgtgcctagcaatcagcaccacagaagcagaagaagcaccatcgagggcggcatcgaaaccgtgaacaatgcttccctgctgaagaccacaagcagcgtggagttcgccatgctgcagttcgcctacgactacatccaagcccacgtgaacgagatgctgagcagaatcgccaccgcctggtgcaccctgcagaacagagagcacgtgctgtggaccgaaaccctgaagctgaaccccggcggcgtggtgagcatggccctggagagaagagtgagcgctagactgctgggcgacgccgtggccgtgacacagtgcgtgaacatcagcagcggccacgtgtacattcagaacagcatgagagtgaccggcagcagcaccacctgctacagcagacccctggtgagcttcagagccctgaacgacagcgagtacatcgaggggcagctgggcgagaacaacgagctgctggtggagagaaagctgatcgagccctgcaccgtgaacaacaagagatacttcaagttcggcgctgactacgtgtacttcgaggactacgcctacgtgagaaaagtgcccctgagcgagatcgagctgatcagcgcctacgtggacctgaacctgaccctgctggaggacagagagttcctgcccctggaggtgtacacaagagccgagctggaggacaccggcctgctggactacagcgagattcagagaagaaatcagctgcacgccctgaagttctacgacatcgacagcatcgtgagagtggacaacaacctggtgatcatgagagggatggccaactttttccaaggcctcggcgacgtcggcgctggcttcggcaaagtggtgctgggcgccgcctccgccgtgatcagcaccgtgagcggcgtgagcagcttcctgaacaaccccttctagtgagctggagcctcggtggcctagcttcttgccccttgggcctccccccagcccctcctccccttcctgcacccgtacccccgtggtctttgaataaagtctgagtgggcggcaaaaaaaaaaaaaaaaaaaaaaaaaa

SEQ ID NO: 6 - RNA, 1186 nt, synthetic construct
  source 1..1186: mol_type = other RNA
gggaaataagagagaaaagaagagtaagaagaaatataagaccccggcgccgccaccatgatgacaagactgcacttctggtggtgcggcatcttcgccgtgctgaagtacctggtgtgcacaagcagcctgaccacaacccccaagaccacaaccgtgtacgtgaagggcttcaacatcccccccctgagatacaactacacccaagctagaatcgtgcccaagatcccccaagccatggaccccaagatcaccgccgaggtgagatacgtgacaagcatggacagctgcggcatggtggccctgatcagcgagcccgacatcgacgctaccatcagaacaattcagctgagccaaaagaagacctacaatgctaccatcagctggttcaaggtgacccaaggctgcgagtaccccatgttcctgatggacatgagactgtgcgaccccaagagagagttcggcatctgcgccctgagaagccctagctactggctggagcccctgaccaagtacatgttcctgaccgacgacgagctgggcctgatcatgatggcccccgctcagttcaaccaagggcagtacagaagagtgatcaccatcgacggcagcatgttctacaccgacttcatggtgcagctgagccccaccccctgctggttcgccaagcccgacagatacgaggagatcctgcacgagtggtgcagaaacgtgaagaccatcggcctggacggcgctagagactaccactactactgggtgccctacaaccctcagccccaccacaaggccgtgctgctgtactggtacagaacccacggcagagagccccccgtgagattccaagaggccatcagatacgacagacccgccatccctagcggcagcgaggacagcaagagaagcaacgacagcagaggcgagagcagcggccccaactggatcgacatcgagaactacacccccaagaacaacgtgcccatcattatcagcgacgatgacgtgcccaccgccccccccaagggcatgaacaatcagagcgtgtagtgagctggagcctcggtggcctagcttcttgccccttgggcctccccccagcccctcctccccttcctgcacccgtacccccgtggtctttgaataaagtctgagtgggcggcaaaaaaaaaaaaaaaaaaaaaaaaaa

SEQ ID NO: 7 - RNA, 1913 nt, synthetic construct
  source 1..1913: mol_type = other RNA
gggaaataagagagaaaagaagagtaagaagaaatataagaccccggcgccgccaccatgggaacacgtctacatttttggtggtgtggaatctttgcggtcctgaaatatctggtatgtacttcaagcgcggatgacgggtcaatcacagcacccgagcaaggaacaatggttggcggcgtcatcgctgaacccagcgcccagatgtcaacagctgctgatatggccaccgggaaaagcgttgattctgagtgggaggcattcttctcctttcacaccagcgtcaattggagtacatctgaaacccaaggaaagattctcttcaaacaatccttaggccctttgctcaacccatatctagaacaccttgctaagctatatgttgcgtggtctgggtcgattgaggttaggttctctatctctggctctggtgtctttggtgggaagctcgcagctattgttgtacctcctggggttgatccagtgcagagtacttcgatgctacaatacccccatgtcttgtttgatgctcgtcaggtggaaccagttatcttctctattcctgatctaagaagcaccctgtaccaccttatgtctgacactgacactacatccttggtcattatggtgtacaatgatctcatcaatccctatgccaatgatgccaactcttctgggtgtattgtcactgtcgagacaaaacctggccctgacttcaagtttcacctccttaagccacccggatctatgctaacccatggttctgtcccttctgatttaattcccaaaacatcttcgctctggatcggtaaccgctactggtcagacataactgattttgtgattcggccgtttgtcttccaagcaaatcgtcattttgactttaatcaagagaccgcagggtggagcacaccacggtttcggcctatatctgttaccattagtgaacagaacggagcaaaattgggcattggagtggcaacagattacatagtgcctggaatccctgatggctggcctgacaccacaattcctggggagttgataccagctggcgattacgcaatcaccaatggtactggcaatgacatcaccacggctacaggatatgacactgctgatataattaagaacaataccaactttaggggcatgtacatatgtggttcgctccagcgtgcctggggtgataagaaaatttccaacactgcctttatcaccactgccaccctagatggtgacaacaacaacaagatcaatccctgtaataccatagaccagtcaaagatcgtcgtgtttcaagacaaccatgttggaaagaaagtgcaaatctcagacgatacattggccctgcttggttacactggcattggtgagcaggccatcgggtctgatagggaccgggttgtgcgcatcagcactctccctgaaactggtgctcgaggcggtaaccacccaattttctacaagaactccattaaattgggatatgtaattaggtctattgatgtctttaattcacaaatcttgcacacttccagacagttatcgctaaatcattacctactcccacttgattcttttgccgtctatagaataattgactcaggtggctcgtggtttgatattggaattgatagtgatgggttctcttttgttggtgtttctggctttggtaaattagaatttcccctttctgcctcctacatgggaatacaattggcaaagatccggcttgcctctaacattaggagtcccatgactaagttagcttaagctggagcctcggtggcctagcttcttgccccttgggcctccccccagcccctcctccccttcctgcacccgtacccccgtggtctttgaataaagtctgagtgggcggcaaaaaaaaaaaaaaaaaaaaaaaaaaa

SEQ ID NO: 8 - RNA, 2018 nt, synthetic construct
  source 1..2018: mol_type = other RNA
gggaaataagagagaaaagaagagtaagaagaaatataagaccccggcgccgccaccatgacacgtctacatttttggtggtgtggaatctttgcggtcctgaaatatctggtatgtacttcaagcagtgatggagcagttcaaccagacggtggtcaacctgctgtcagaaatgaaagagctacaggatctgggaacgggtctggaggcgggggtggtggtggttctgggggtgtggggatttctacgggtactttcaataatcagacggaatttaaatttttggaaaacggatgggtggaaatcacagcaaactcaagcagacttgtacatttaaatatgccagaaagtgaaaattataaaagagtagttgtaaataatatggataaaactgcagttaaaggaaacatggctttagatgatactcatgtacaaattgtaactccttggtcattggttgatgcaaatgcttggggagtttggtttaatccaggagattggcaactaattgttaatactatgagtgagttgcatttagttagttttgaacaagaaatttttaatgttgttttaaagactgtttcagaatctgctactcagccaccaactaaagtttataataatgatttaactgcatcattgatggttgcattagatagtaataatactatgccatttactccagcagctatgagatctgagacattgggtttttatccatggaaaccaaccataccaactccatggagatattattttcaatgggatagaacattaataccatctcatactggaactagtggcacaccaacaaatgtatattatggtacagatccagatgatgttcaattttatactattgaaaattctgtgccagtacacttactaagaacaggtgatgaatttgctacaggaacatttttttttgattgtaaaccatgtagactaacacatacatggcaaacaaatagagcattgggcttaccaccatttctaaattctttgcctcaatctgaaggagctactaactttggtgatataggagttcaacaagataaaagacgtggtgtaactcaaatgggaaatacagactatattactgaagctactattatgagaccagctgaggttggttatagtgcaccatattattcttttgaagcatctacacaagggccatttaaaacacctattgcagcaggacgggggggagcgcaaacagatgaaaatcaagcagcagatggtgatccaagatatgcatttggtagacaacatggtcaaaaaactactacaacaggagaaacacccgagagattgacatatatagcacatcaagatacaggaagatatccagaaggagattggattcaaaatattaactttaaccttcctgtaacaaatgataatgtattgctaccaacagatccaattggaggtaaaacaggaattaactatactaatatatttaatacttatggtcctttaactgcattaaataatgtaccaccagtttatccaaatggtcaaatttgggataaagaatttgatactgacttaaaaccaagacttcatgtaaatgcaccatttgtttgtcaaaataattgtcctggtcaattatttgtaaaagttgcgcctaatttaacaaatgaatatgatcctgatgcatctgctaatatgtcaagaattgtaacttactcagatttttggtggaaaggtaaattagtatttaaagctaaactaagagcatctcatacttggaatccaattcaacaaatgagtattaatgtagataaccaatttaactatgtaccaaataatattggagctatgaaaattgtatatgaaaaatctcaactagcacctagaaaattatattagtgagctggagcctcggtggcctagcttcttgccccttgggcctccccccagcccctcctccccttcctgcacccgtacccccgtggtctttgaataaagtctgagtgggcggcaaaaaaaaaaaaaaaaaaaaaaaaaaa

SEQ ID NO: 9 - RNA, 10215 nt, synthetic construct
  source 1..10215: mol_type = other RNA
atgggcggcgcatgagagaagcccagaccaattacctacccaaaatggagaaagttcacgttgacatcgaggaagacagcccattcctcagagctttgcagcggagcttcccgcagtttgaggtagaagccaagcaggtcactgataatgaccatgctaatgccagagcgttttcgcatctggcttcaaaactgatcgaaacggaggtggacccatccgacacgatccttgacattggaagtgcgcccgcccgcagaatgtattctaagcacaagtatcattgtatctgtccgatgagatgtgcggaagatccggacagattgtataagtatgcaactaagctgaagaaaaactgtaaggaaataactgataaggaattggacaagaaaatgaaggagctggccgccgtcatgagcgaccctgacctggaaactgagactatgtgcctccacgacgacgagtcgtgtcgctacgaagggcaagtcgctgtttaccaggatgtatacgcggttgacggaccgacaagtctctatcaccaagccaataagggagttagagtcgcctactggataggctttgacaccaccccttttatgtttaagaacttggctggagcatatccatcatactctaccaactgggccgacgaaaccgtgttaacggctcgtaacataggcctatgcagctctgacgttatggagcggtcacgtagagggatgtccattcttagaaagaagtatttgaaaccatccaacaatgttctattctctgttggctcgaccatctaccacgagaagagggacttactgaggagctggcacctgccgtctgtatttcacttacgtggcaagcaaaattacacatgtcggtgtgagactatagttagttgcgacgggtacgtcgttaaaagaatagctatcagtccaggcctgtatgggaagccttcaggctatgctgctacgatgcaccgcgagggattcttgtgctgcaaagtgacagacacattgaacggggagagggtctcttttcccgtgtgcacgtatgtgccagctacattgtgtgaccaaatgactggcatactggcaacagatgtcagtgcggacgacgcgcaaaaactgctggttgggctcaaccagcgtatagtcgtcaacggtcgcacccagagaaacaccaataccatgaaaaattaccttttgcccgtagtggcccaggcatttgctaggtgggcaaaggaatataaggaagatcaagaagatgaaaggccactaggactacgagatagacagttagtcatggggtgttgttgggcttttagaaggcacaagataacatctatttataagcgcccggatacccaaaccatcatcaaagtgaacagcgatttccactcattcgtgctgcccaggataggcagtaacacattggagatcgggctgagaacaagaatcaggaaaatgttagaggagcacaaggagccgtcacctctcattaccgccgaggacgtacaagaagctaagtgcgcagccgatgaggctaaggaggtgcgtgaagccgaggagttgcgcgcagctctaccacctttggcagctgatgttgaggagcccactctggaggcagacgtcgacttgatgttacaagaggctggggccggctcagtggagacacctcgtggcttgataaaggttaccagctacgatggcgaggacaagatcggctcttacgctgtgctttctccgcaggctgtactcaagagtgaaaaattatcttgcatccaccctctcgctgaacaagtcatagtgataacacactctggccgaaaagggcgttatgccgtggaaccataccatggtaaagtagtggtgccagagggacatgcaatacccgtccaggactttcaagctctgagtgaaagtgccaccattgtgtacaacgaacgtgagttcgtaaacaggtacctgcaccatattgccacacatggaggagcgctgaacactgatgaagaatattacaaaactgtcaagcccagcgagcacgacggcgaatacctgtacgacatcgacaggaaacagtgcgtcaagaaagaactagtcactgggctagggctcacaggcgagctggtggatcctcccttccatgaattcgcctacgagagtctgagaacacgaccagccgctccttaccaagtaccaaccataggggtgtatggcgtgccaggatcaggcaagtctggcatcattaaaagcgcagtcaccaaaaaagatctagtggtgagcgccaagaaagaaaactgtgcagaaattataagggacgtcaagaaaatgaaagggctggacgtcaatgccagaactgtggactcagtgctcttgaatggatgcaaacaccccgtagagaccctgtatattgacgaagcttttgcttgtcatgcaggtactctcagagcgctcatagccattataagacctaaaaaggcagtgctctgcggggatcccaaacagtgcggtttttttaacatgatgtgcctgaaagtgcattttaaccacgagatttgcacacaagtcttccacaaaagcatctctcgccgttgcactaaatctgtgacttcggtcgtctcaaccttgttttacgacaaaaaaatgagaacgacgaatccgaaagagactaagattgtgattgacactaccggcagtaccaaacctaagcaggacgatctcattctcacttgtttcagagggtgggtgaagcagttgcaaatagattacaaaggcaacgaaataatgacggcagctgcctctcaagggctgacccgtaaaggtgtgtatgccgttcggtacaaggtgaatgaaaatcctctgtacgcacccacctcagaacatgtgaacgtcctactgacccgcacggaggaccgcatcgtgtggaaaacactagccggcgacccatggataaaaacactgactgccaagtaccctgggaatttcactgccacgatagaggagtggcaagcagagcatgatgccatcatgaggcacatcttggagagaccggaccctaccgacgtcttccagaataaggcaaacgtgtgttgggccaaggctttagtgccggtgctgaagaccgctggcatagacatgaccactgaacaatggaacactgtggattattttgaaacggacaaagctcactcagcagagatagtattgaaccaactatgcgtgaggttctttggactcgatctggactccggtctattttctgcacccactgttccgttatccattaggaataatcactgggataactccccgtcgcctaacatgtacgggctgaataaagaagtggtccgtcagctctctcgcaggtacccacaactgcctcgggcagttgccactggaagagtctatgacatgaacactggtacactgcgcaattatgatccgcgcataaacctagtacctgtaaacagaagactgcctcatgctttagtcctccaccataatgaacacccacagagtgacttttcttcattcgtcagcaaattgaagggcagaactgtcctggtggtcggggaaaagttgtccgtcccaggcaaaatggttgactggttgtcagaccggcctgaggctaccttcagagctcggctggatttaggcatcccaggtgatgtgcccaaatatgacataatatttgttaatgtgaggaccccatataaataccatcactatcagcagtgtgaagaccatgccattaagcttagcatgttgaccaagaaagcttgtctgcatctgaatcccggcggaacctgtgtcagcataggttatggttacgctgacagggccagcgaaagcatcattggtgctatagcgcggcagttcaagttttcccgggtatgcaaaccgaaatcctcacttgaagagacggaagttctgtttgtattcattgggtacgatcgcaaggcccgtacgcacaattcttacaagctttcatcaaccttgaccaacatttatacaggttccagactccacgaagccggatgtgcaccctcatatcatgtggtgcgaggggatattgccacggccaccgaaggagtgattataaatgctgctaacagcaaaggacaacctggcggaggggtgtgcggagcgctgtataagaaattcccggaaagcttcgatttacagccgatcgaagtaggaaaagcgcgactggtcaaaggtgcagctaaacatatcattcatgccgtaggaccaaacttcaacaaagtttcggaggttgaaggtgacaaacagttggcagaggcttatgagtccatcgctaagattgtcaacgataacaattacaagtcagtagcgattccactgttgtccaccggcatcttttccgggaacaaagatcgactaacccaatcattgaaccatttgctgacagctttagacaccactgatgcagatgtagccatatactgcagggacaagaaatgggaaatgactctcaaggaagcagtggctaggagagaagcagtggaggagatatgcatatccgacgactcttcagtgacagaacctgatgcagagctggtgagggtgcatccgaagagttctttggctggaaggaagggctacagcacaagcgatggcaaaactttctcatatttggaagggaccaagtttcaccaggcggccaaggatatagcagaaattaatgccatgtggcccgttgcaacggaggccaatgagcaggtatgcatgtatatcctcggagaaagcatgagcagtattaggtcgaaatgccccgtcgaagagtcggaagcctccacaccacctagcacgctgccttgcttgtgcatccatgccatgactccagaaagagtacagcgcctaaaagcctcacgtccagaacaaattactgtgtgctcatcctttccattgccgaagtatagaatcactggtgtgcagaagatccaatgctcccagcctatattgttctcaccgaaagtgcctgcgtatattcatccaaggaagtatctcgtggaaacaccaccggtagacgagactccggagccatcggcagagaaccaatccacagaggggacacctgaacaaccaccacttataaccgaggatgagaccaggactagaacgcctgagccgatcatcatcgaagaggaagaagaggatagcataagtttgctgtcagatggcccgacccaccaggtgctgcaagtcgaggcagacattcacgggccgccctctgtatctagctcatcctggtccattcctcatgcatccgactttgatgtggacagtttatccatacttgacaccctggagggagctagcgtgaccagcggggcaacgtcagccgagactaactcttacttcgcaaagagtatggagtttctggcgcgaccggtgcctgcgcctcgaacagtattcaggaaccctccacatcccgctccgcgcacaagaacaccgtcacttgcacccagcagggcctgctcgagaaccagcctagtttccaccccgccaggcgtgaatagggtgatcactagagaggagctcgaggcgcttaccccgtcacgcactcctagcaggtcggtctcgagaaccagcctggtctccaacccgccaggcgtaaatagggtgattacaagagaggagtttgaggcgttcgtagcacaacaacaatgacggtttgatgcgggtgcatacatcttttcctccgacaccggtcaagggcatttacaacaaaaatcagtaaggcaaacggtgctatccgaagtggtgttggagaggaccgaattggagatttcgtatgccccgcgcctcgaccaagaaaaagaagaattactacgcaagaaattacagttaaatcccacacctgctaacagaagcagataccagtccaggaaggtggagaacatgaaagccataacagctagacgtattctgcaaggcctagggcattatttgaaggcagaaggaaaagtggagtgctaccgaaccctgcatcctgttcctttgtattcatctagtgtgaaccgtgccttttcaagccccaaggtcgcagtggaagcctgtaacgccatgttgaaagagaactttccgactgtggcttcttactgtattattccagagtacgatgcctatttggacatggttgacggagcttcatgctgcttagacactgccagtttttgccctgcaaagctgcgcagctttccaaagaaacactcctatttggaacccacaatacgatcggcagtgccttcagcgatccagaacacgctccagaacgtcctggcagctgccacaaaaagaaattgcaatgtcacgcaaatgagagaattgcccgtattggattcggcggcctttaatgtggaatgcttcaagaaatatgcgtgtaataatgaatattgggaaacgtttaaagaaaaccccatcaggcttactgaagaaaacgtggtaaattacattaccaaattaaaaggaccaaaagctgctgctctttttgcgaagacacataatttgaatatgttgcaggacataccaatggacaggtttgtaatggacttaaagagagacgtgaaagtgactccaggaacaaaacatactgaagaacggcccaaggtacaggtgatccaggctgccgatccgctagcaacagcgtatctgtgcggaatccaccgagagctggttaggagattaaatgcggtcctgcttccgaacattcatacactgtttgatatgtcggctgaagactttgacgctattatagccgagcacttccagcctggggattgtgttctggaaactgacatcgcgtcgtttgataaaagtgaggacgacgccatggctctgaccgcgttaatgattctggaagacttaggtgtggacgcagagctgttgacgctgattgaggcggctttcggcgaaatttcatcaatacatttgcccactaaaactaaatttaaattcggagccatgatgaaatctggaatgttcctcacactgtttgtgaacacagtcattaacattgtaatcgcaagcagagtgttgagagaacggctaaccggatcaccatgtgcagcattcattggagatgacaatatcgtgaaaggagtcaaatcggacaaattaatggcagacaggtgcgccacctggttgaatatggaagtcaagattatagatgctgtggtgggcgagaaagcgccttatttctgtggagggtttattttgtgtgactccgtgaccggcacagcgtgccgtgtggcagaccccctaaaaaggctgtttaagcttggcaaacctctggcagcagacgatgaacatgatgatgacaggagaagggcattgcatgaagagtcaacacgctggaaccgagtgggtattctttcagagctgtgcaaggcagtagaatcaaggtatgaaaccgtaggaacttccatcatagttatggccatgactactctagctagcagtgttaaatcattcagctacctgagaggggcccctataactctctacggctaacctgaatggactacgacatagtctagtccgccaagtctagcatatgatgacaagactgcacttctggtggtgcggcatcttcgccgtgctgaagtacctggtgtgcacaagcagcagcacccggggcgacctgggcaagagacggagaggcagcagatggcaaggccacagcggctacttcagacagagatgcttcttccctagcctgctgggcatcgccgccaccggcagcagacacggcaacggcagcagcggcctgacaagactggctagatacgtgagcttcatctggatcgtgctgttcctggtgggccctagacccgtggaggggcagagcggcagcacaagcgaacagcctagaagaaccgtggccacccccgaggtcggcggcaccccccccaagcccaccaccgaccccaccgacatgtccgacatgagagaggccctgagagctagccaaatcgaggccaacggccctagcaccttctacatgtgcccccctccctccggcagcaccgtggtgagactggagccccctagagcctgccccgactacaagctgggcaagaacttcaccgagggcatcgccgtgatcttcaaggagaacatcgccccctacaagttcaaggccaacatctactacaagaacatcatcatgaccaccgtgtggagcggcagcagctacgccgtgaccaccaacagatacaccgacagagtgcccgtgaaggtgcaagagatcaccgacctgatcgacagaagaggcatgtgcctgagcaaggccgattacgtgagaaacaactatcagttcaccgccttcgacagagacgaggaccctagagagctgcccctgaagcctagcaagttcaacacccccgagagcagaggctggcacaccaccaacgaaacctacaccaagatcggcgccgccggcttccaccacagcggcacaagcgtgaactgcatcgtggaagaggtggacgctagaagcgtgtacccctacgacagcttcgccatctccaccggcgacgtgattcacatgagccccttcttcggcctgagagacggcgcccacgtggagcacacaagctacagcagcgacagatttcagcagatcgagggctactaccccatcgacctggacacaagactgcagctgggcgcccccgtgagcagaaacttcctggaaaccccccacgtgaccgtggcctggaactggacccccaagagcggcagagtgtgcaccctggccaagtggagagagatcgacgaaatgctgagagacgagtaccaaggcagctacagattcaccgccaagaccatcagcgccaccttcatcagcaacacaagccaattcgagatcaacagaatcagactgggcgactgcgccaccaaggaggccgccgaggccatcgacagaatctacaagagcaagtacagcaagacccacattcagaccggcaccctggaaacctacctggctagaggcggcttcctgatcgccttcagacccatgatcagcaatgagctggccaagctgtacatcaacgagctggctagaagcaacagaaccgtggacctgagcgccctgctgaaccctagcggcgaaaccgtgcagagaacaagaagaagcgtgcctagcaatcagcaccacagaagcagaagaagcaccatcgagggcggcatcgaaaccgtgaacaatgcttccctgctgaagaccacaagcagcgtggagttcgccatgctgcagttcgcctacgactacatccaagcccacgtgaacgagatgctgagcagaatcgccaccgcctggtgcaccctgcagaacagagagcacgtgctgtggaccgaaaccctgaagctgaaccccggcggcgtggtgagcatggccctggagagaagagtgagcgctagactgctgggcgacgccgtggccgtgacacagtgcgtgaacatcagcagcggccacgtgtacattcagaacagcatgagagtgaccggcagcagcaccacctgctacagcagacccctggtgagcttcagagccctgaacgacagcgagtacatcgaggggcagctgggcgagaacaacgagctgctggtggagagaaagctgatcgagccctgcaccgtgaacaacaagagatacttcaagttcggcgctgactacgtgtacttcgaggactacgcctacgtgagaaaagtgcccctgagcgagatcgagctgatcagcgcctacgtggacctgaacctgaccctgctggaggacagagagttcctgcccctggaggtgtacacaagagccgagctggaggacaccggcctgctggactacagcgagattcagagaagaaatcagctgcacgccctgaagttctacgacatcgacagcatcgtgagagtggacaacaacctggtgatcatgagagggatggccaactttttccaaggcctcggcgacgtcggcgctggcttcggcaaagtggtgctgggcgccgcctccgccgtgatcagcaccgtgagcggcgtgagcagcttcctgaacaaccccttctaggaattggcaagctgcttacatagaactcgcggcgattggcatgccgccttaaaatttttattttattttttcttttcttttccgaatcggattttgtttttaatatttcaaaaaaaaaaaaaaaaaaaaaaaaaa

SEQ ID NO: 10 - RNA, 8697 nt, synthetic construct
  source 1..8697: mol_type = other RNA
atgggcggcgcatgagagaagcccagaccaattacctacccaaaatggagaaagttcacgttgacatcgaggaagacagcccattcctcagagctttgcagcggagcttcccgcagtttgaggtagaagccaagcaggtcactgataatgaccatgctaatgccagagcgttttcgcatctggcttcaaaactgatcgaaacggaggtggacccatccgacacgatccttgacattggaagtgcgcccgcccgcagaatgtattctaagcacaagtatcattgtatctgtccgatgagatgtgcggaagatccggacagattgtataagtatgcaactaagctgaagaaaaactgtaaggaaataactgataaggaattggacaagaaaatgaaggagctggccgccgtcatgagcgaccctgacctggaaactgagactatgtgcctccacgacgacgagtcgtgtcgctacgaagggcaagtcgctgtttaccaggatgtatacgcggttgacggaccgacaagtctctatcaccaagccaataagggagttagagtcgcctactggataggctttgacaccaccccttttatgtttaagaacttggctggagcatatccatcatactctaccaactgggccgacgaaaccgtgttaacggctcgtaacataggcctatgcagctctgacgttatggagcggtcacgtagagggatgtccattcttagaaagaagtatttgaaaccatccaacaatgttctattctctgttggctcgaccatctaccacgagaagagggacttactgaggagctggcacctgccgtctgtatttcacttacgtggcaagcaaaattacacatgtcggtgtgagactatagttagttgcgacgggtacgtcgttaaaagaatagctatcagtccaggcctgtatgggaagccttcaggctatgctgctacgatgcaccgcgagggattcttgtgctgcaaagtgacagacacattgaacggggagagggtctcttttcccgtgtgcacgtatgtgccagctacattgtgtgaccaaatgactggcatactggcaacagatgtcagtgcggacgacgcgcaaaaactgctggttgggctcaaccagcgtatagtcgtcaacggtcgcacccagagaaacaccaataccatgaaaaattaccttttgcccgtagtggcccaggcatttgctaggtgggcaaaggaatataaggaagatcaagaagatgaaaggccactaggactacgagatagacagttagtcatggggtgttgttgggcttttagaaggcacaagataacatctatttataagcgcccggatacccaaaccatcatcaaagtgaacagcgatttccactcattcgtgctgcccaggataggcagtaacacattggagatcgggctgagaacaagaatcaggaaaatgttagaggagcacaaggagccgtcacctctcattaccgccgaggacgtacaagaagctaagtgcgcagccgatgaggctaaggaggtgcgtgaagccgaggagttgcgcgcagctctaccacctttggcagctgatgttgaggagcccactctggaggcagacgtcgacttgatgttacaagaggctggggccggctcagtggagacacctcgtggcttgataaaggttaccagctacgatggcgaggacaagatcggctcttacgctgtgctttctccgcaggctgtactcaagagtgaaaaattatcttgcatccaccctctcgctgaacaagtcatagtgataacacactctggccgaaaagggcgttatgccgtggaaccataccatggtaaagtagtggtgccagagggacatgcaatacccgtccaggactttcaagctctgagtgaaagtgccaccattgtgtacaacgaacgtgagttcgtaaacaggtacctgcaccatattgccacacatggaggagcgctgaacactgatgaagaatattacaaaactgtcaagcccagcgagcacgacggcgaatacctgtacgacatcgacaggaaacagtgcgtcaagaaagaactagtcactgggctagggctcacaggcgagctggtggatcctcccttccatgaattcgcctacgagagtctgagaacacgaccagccgctccttaccaagtaccaaccataggggtgtatggcgtgccaggatcaggcaagtctggcatcattaaaagcgcagtcaccaaaaaagatctagtggtgagcgccaagaaagaaaactgtgcagaaattataagggacgtcaagaaaatgaaagggctggacgtcaatgccagaactgtggactcagtgctcttgaatggatgcaaacaccccgtagagaccctgtatattgacgaagcttttgcttgtcatgcaggtactctcagagcgctcatagccattataagacctaaaaaggcagtgctctgcggggatcccaaacagtgcggtttttttaacatgatgtgcctgaaagtgcattttaaccacgagatttgcacacaagtcttccacaaaagcatctctcgccgttgcactaaatctgtgacttcggtcgtctcaaccttgttttacgacaaaaaaatgagaacgacgaatccgaaagagactaagattgtgattgacactaccggcagtaccaaacctaagcaggacgatctcattctcacttgtttcagagggtgggtgaagcagttgcaaatagattacaaaggcaacgaaataatgacggcagctgcctctcaagggctgacccgtaaaggtgtgtatgccgttcggtacaaggtgaatgaaaatcctctgtacgcacccacctcagaacatgtgaacgtcctactgacccgcacggaggaccgcatcgtgtggaaaacactagccggcgacccatggataaaaacactgactgccaagtaccctgggaatttcactgccacgatagaggagtggcaagcagagcatgatgccatcatgaggcacatcttggagagaccggaccctaccgacgtcttccagaataaggcaaacgtgtgttgggccaaggctttagtgccggtgctgaagaccgctggcatagacatgaccactgaacaatggaacactgtggattattttgaaacggacaaagctcactcagcagagatagtattgaaccaactatgcgtgaggttctttggactcgatctggactccggtctattttctgcacccactgttccgttatccattaggaataatcactgggataactccccgtcgcctaacatgtacgggctgaataaagaagtggtccgtcagctctctcgcaggtacccacaactgcctcgggcagttgccactggaagagtctatgacatgaacactggtacactgcgcaattatgatccgcgcataaacctagtacctgtaaacagaagactgcctcatgctttagtcctccaccataatgaacacccacagagtgacttttcttcattcgtcagcaaattgaagggcagaactgtcctggtggtcggggaaaagttgtccgtcccaggcaaaatggttgactggttgtcagaccggcctgaggctaccttcagagctcggctggatttaggcatcccaggtgatgtgcccaaatatgacataatatttgttaatgtgaggaccccatataaataccatcactatcagcagtgtgaagaccatgccattaagcttagcatgttgaccaagaaagcttgtctgcatctgaatcccggcggaacctgtgtcagcataggttatggttacgctgacagggccagcgaaagcatcattggtgctatagcgcggcagttcaagttttcccgggtatgcaaaccgaaatcctcacttgaagagacggaagttctgtttgtattcattgggtacgatcgcaaggcccgtacgcacaattcttacaagctttcatcaaccttgaccaacatttatacaggttccagactccacgaagccggatgtgcaccctcatatcatgtggtgcgaggggatattgccacggccaccgaaggagtgattataaatgctgctaacagcaaaggacaacctggcggaggggtgtgcggagcgctgtataagaaattcccggaaagcttcgatttacagccgatcgaagtaggaaaagcgcgactggtcaaaggtgcagctaaacatatcattcatgccgtaggaccaaacttcaacaaagtttcggaggttgaaggtgacaaacagttggcagaggcttatgagtccatcgctaagattgtcaacgataacaattacaagtcagtagcgattccactgttgtccaccggcatcttttccgggaacaaagatcgactaacccaatcattgaaccatttgctgacagctttagacaccactgatgcagatgtagccatatactgcagggacaagaaatgggaaatgactctcaaggaagcagtggctaggagagaagcagtggaggagatatgcatatccgacgactcttcagtgacagaacctgatgcagagctggtgagggtgcatccgaagagttctttggctggaaggaagggctacagcacaagcgatggcaaaactttctcatatttggaagggaccaagtttcaccaggcggccaaggatatagcagaaattaatgccatgtggcccgttgcaacggaggccaatgagcaggtatgcatgtatatcctcggagaaagcatgagcagtattaggtcgaaatgccccgtcgaagagtcggaagcctccacaccacctagcacgctgccttgcttgtgcatccatgccatgactccagaaagagtacagcgcctaaaagcctcacgtccagaacaaattactgtgtgctcatcctttccattgccgaagtatagaatcactggtgtgcagaagatccaatgctcccagcctatattgttctcaccgaaagtgcctgcgtatattcatccaaggaagtatctcgtggaaacaccaccggtagacgagactccggagccatcggcagagaaccaatccacagaggggacacctgaacaaccaccacttataaccgaggatgagaccaggactagaacgcctgagccgatcatcatcgaagaggaagaagaggatagcataagtttgctgtcagatggcccgacccaccaggtgctgcaagtcgaggcagacattcacgggccgccctctgtatctagctcatcctggtccattcctcatgcatccgactttgatgtggacagtttatccatacttgacaccctggagggagctagcgtgaccagcggggcaacgtcagccgagactaactcttacttcgcaaagagtatggagtttctggcgcgaccggtgcctgcgcctcgaacagtattcaggaaccctccacatcccgctccgcgcacaagaacaccgtcacttgcacccagcagggcctgctcgagaaccagcctagtttccaccccgccaggcgtgaatagggtgatcactagagaggagctcgaggcgcttaccccgtcacgcactcctagcaggtcggtctcgagaaccagcctggtctccaacccgccaggcgtaaatagggtgattacaagagaggagtttgaggcgttcgtagcacaacaacaatgacggtttgatgcgggtgcatacatcttttcctccgacaccggtcaagggcatttacaacaaaaatcagtaaggcaaacggtgctatccgaagtggtgttggagaggaccgaattggagatttcgtatgccccgcgcctcgaccaagaaaaagaagaattactacgcaagaaattacagttaaatcccacacctgctaacagaagcagataccagtccaggaaggtggagaacatgaaagccataacagctagacgtattctgcaaggcctagggcattatttgaaggcagaaggaaaagtggagtgctaccgaaccctgcatcctgttcctttgtattcatctagtgtgaaccgtgccttttcaagccccaaggtcgcagtggaagcctgtaacgccatgttgaaagagaactttccgactgtggcttcttactgtattattccagagtacgatgcctatttggacatggttgacggagcttcatgctgcttagacactgccagtttttgccctgcaaagctgcgcagctttccaaagaaacactcctatttggaacccacaatacgatcggcagtgccttcagcgatccagaacacgctccagaacgtcctggcagctgccacaaaaagaaattgcaatgtcacgcaaatgagagaattgcccgtattggattcggcggcctttaatgtggaatgcttcaagaaatatgcgtgtaataatgaatattgggaaacgtttaaagaaaaccccatcaggcttactgaagaaaacgtggtaaattacattaccaaattaaaaggaccaaaagctgctgctctttttgcgaagacacataatttgaatatgttgcaggacataccaatggacaggtttgtaatggacttaaagagagacgtgaaagtgactccaggaacaaaacatactgaagaacggcccaaggtacaggtgatccaggctgccgatccgctagcaacagcgtatctgtgcggaatccaccgagagctggttaggagattaaatgcggtcctgcttccgaacattcatacactgtttgatatgtcggctgaagactttgacgctattatagccgagcacttccagcctggggattgtgttctggaaactgacatcgcgtcgtttgataaaagtgaggacgacgccatggctctgaccgcgttaatgattctggaagacttaggtgtggacgcagagctgttgacgctgattgaggcggctttcggcgaaatttcatcaatacatttgcccactaaaactaaatttaaattcggagccatgatgaaatctggaatgttcctcacactgtttgtgaacacagtcattaacattgtaatcgcaagcagagtgttgagagaacggctaaccggatcaccatgtgcagcattcattggagatgacaatatcgtgaaaggagtcaaatcggacaaattaatggcagacaggtgcgccacctggttgaatatggaagtcaagattatagatgctgtggtgggcgagaaagcgccttatttctgtggagggtttattttgtgtgactccgtgaccggcacagcgtgccgtgtggcagaccccctaaaaaggctgtttaagcttggcaaacctctggcagcagacgatgaacatgatgatgacaggagaagggcattgcatgaagagtcaacacgctggaaccgagtgggtattctttcagagctgtgcaaggcagtagaatcaaggtatgaaaccgtaggaacttccatcatagttatggccatgactactctagctagcagtgttaaatcattcagctacctgagaggggcccctataactctctacggctaacctgaatggactacgacatagtctagtccgccaagtctagcatatgatgatgacaagactgcacttctggtggtgcggcatcttcgccgtgctgaagtacctggtgtgcacaagcagcctgaccacaacccccaagaccacaaccgtgtacgtgaagggcttcaacatcccccccctgagatacaactacacccaagctagaatcgtgcccaagatcccccaagccatggaccccaagatcaccgccgaggtgagatacgtgacaagcatggacagctgcggcatggtggccctgatcagcgagcccgacatcgacgctaccatcagaacaattcagctgagccaaaagaagacctacaatgctaccatcagctggttcaaggtgacccaaggctgcgagtaccccatgttcctgatggacatgagactgtgcgaccccaagagagagttcggcatctgcgccctgagaagccctagctactggctggagcccctgaccaagtacatgttcctgaccgacgacgagctgggcctgatcatgatggcccccgctcagttcaaccaagggcagtacagaagagtgatcaccatcgacggcagcatgttctacaccgacttcatggtgcagctgagccccaccccctgctggttcgccaagcccgacagatacgaggagatcctgcacgagtggtgcagaaacgtgaagaccatcggcctggacggcgctagagactaccactactactgggtgccctacaaccctcagccccaccacaaggccgtgctgctgtactggtacagaacccacggcagagagccccccgtgagattccaagaggccatcagatacgacagacccgccatccctagcggcagcgaggacagcaagagaagcaacgacagcagaggcgagagcagcggccccaactggatcgacatcgagaactacacccccaagaacaacgtgcccatcattatcagcgacgatgacgtgcccaccgccccccccaagggcatgaacaatcagagcgtgtaggaattggcaagctgcttacatagaactcgcggcgattggcatgccgccttaaaatttttattttattttttcttttcttttccgaatcggattttgtttttaatatttcaaaaaaaaaaaaaaaaaaaaaaaaaa

SEQ ID NO: 11 - RNA, 9426 nt, synthetic construct
  source 1..9426: mol_type = other RNA
atgggcggcgcatgagagaagcccagaccaattacctacccaaaatggagaaagttcacgttgacatcgaggaagacagcccattcctcagagctttgcagcggagcttcccgcagtttgaggtagaagccaagcaggtcactgataatgaccatgctaatgccagagcgttttcgcatctggcttcaaaactgatcgaaacggaggtggacccatccgacacgatccttgacattggaagtgcgcccgcccgcagaatgtattctaagcacaagtatcattgtatctgtccgatgagatgtgcggaagatccggacagattgtataagtatgcaactaagctgaagaaaaactgtaaggaaataactgataaggaattggacaagaaaatgaaggagctggccgccgtcatgagcgaccctgacctggaaactgagactatgtgcctccacgacgacgagtcgtgtcgctacgaagggcaagtcgctgtttaccaggatgtatacgcggttgacggaccgacaagtctctatcaccaagccaataagggagttagagtcgcctactggataggctttgacaccaccccttttatgtttaagaacttggctggagcatatccatcatactctaccaactgggccgacgaaaccgtgttaacggctcgtaacataggcctatgcagctctgacgttatggagcggtcacgtagagggatgtccattcttagaaagaagtatttgaaaccatccaacaatgttctattctctgttggctcgaccatctaccacgagaagagggacttactgaggagctggcacctgccgtctgtatttcacttacgtggcaagcaaaattacacatgtcggtgtgagactatagttagttgcgacgggtacgtcgttaaaagaatagctatcagtccaggcctgtatgggaagccttcaggctatgctgctacgatgcaccgcgagggattcttgtgctgcaaagtgacagacacattgaacggggagagggtctcttttcccgtgtgcacgtatgtgccagctacattgtgtgaccaaatgactggcatactggcaacagatgtcagtgcggacgacgcgcaaaaactgctggttgggctcaaccagcgtatagtcgtcaacggtcgcacccagagaaacaccaataccatgaaaaattaccttttgcccgtagtggcccaggcatttgctaggtgggcaaaggaatataaggaagatcaagaagatgaaaggccactaggactacgagatagacagttagtcatggggtgttgttgggcttttagaaggcacaagataacatctatttataagcgcccggatacccaaaccatcatcaaagtgaacagcgatttccactcattcgtgctgcccaggataggcagtaacacattggagatcgggctgagaacaagaatcaggaaaatgttagaggagcacaaggagccgtcacctctcattaccgccgaggacgtacaagaagctaagtgcgcagccgatgaggctaaggaggtgcgtgaagccgaggagttgcgcgcagctctaccacctttggcagctgatgttgaggagcccactctggaggcagacgtcgacttgatgttacaagaggctggggccggctcagtggagacacctcgtggcttgataaaggttaccagctacgatggcgaggacaagatcggctcttacgctgtgctttctccgcaggctgtactcaagagtgaaaaattatcttgcatccaccctctcgctgaacaagtcatagtgataacacactctggccgaaaagggcgttatgccgtggaaccataccatggtaaagtagtggtgccagagggacatgcaatacccgtccaggactttcaagctctgagtgaaagtgccaccattgtgtacaacgaacgtgagttcgtaaacaggtacctgcaccatattgccacacatggaggagcgctgaacactgatgaagaatattacaaaactgtcaagcccagcgagcacgacggcgaatacctgtacgacatcgacaggaaacagtgcgtcaagaaagaactagtcactgggctagggctcacaggcgagctggtggatcctcccttccatgaattcgcctacgagagtctgagaacacgaccagccgctccttaccaagtaccaaccataggggtgtatggcgtgccaggatcaggcaagtctggcatcattaaaagcgcagtcaccaaaaaagatctagtggtgagcgccaagaaagaaaactgtgcagaaattataagggacgtcaagaaaatgaaagggctggacgtcaatgccagaactgtggactcagtgctcttgaatggatgcaaacaccccgtagagaccctgtatattgacgaagcttttgcttgtcatgcaggtactctcagagcgctcatagccattataagacctaaaaaggcagtgctctgcggggatcccaaacagtgcggtttttttaacatgatgtgcctgaaagtgcattttaaccacgagatttgcacacaagtcttccacaaaagcatctctcgccgttgcactaaatctgtgacttcggtcgtctcaaccttgttttacgacaaaaaaatgagaacgacgaatccgaaagagactaagattgtgattgacactaccggcagtaccaaacctaagcaggacgatctcattctcacttgtttcagagggtgggtgaagcagttgcaaatagattacaaaggcaacgaaataatgacggcagctgcctctcaagggctgacccgtaaaggtgtgtatgccgttcggtacaaggtgaatgaaaatcctctgtacgcacccacctcagaacatgtgaacgtcctactgacccgcacggaggaccgcatcgtgtggaaaacactagccggcgacccatggataaaaacactgactgccaagtaccctgggaatttcactgccacgatagaggagtggcaagcagagcatgatgccatcatgaggcacatcttggagagaccggaccctaccgacgtcttccagaataaggcaaacgtgtgttgggccaaggctttagtgccggtgctgaagaccgctggcatagacatgaccactgaacaatggaacactgtggattattttgaaacggacaaagctcactcagcagagatagtattgaaccaactatgcgtgaggttctttggactcgatctggactccggtctattttctgcacccactgttccgttatccattaggaataatcactgggataactccccgtcgcctaacatgtacgggctgaataaagaagtggtccgtcagctctctcgcaggtacccacaactgcctcgggcagttgccactggaagagtctatgacatgaacactggtacactgcgcaattatgatccgcgcataaacctagtacctgtaaacagaagactgcctcatgctttagtcctccaccataatgaacacccacagagtgacttttcttcattcgtcagcaaattgaagggcagaactgtcctggtggtcggggaaaagttgtccgtcccaggcaaaatggttgactggttgtcagaccggcctgaggctaccttcagagctcggctggatttaggcatcccaggtgatgtgcccaaatatgacataatatttgttaatgtgaggaccccatataaataccatcactatcagcagtgtgaagaccatgccattaagcttagcatgttgaccaagaaagcttgtctgcatctgaatcccggcggaacctgtgtcagcataggttatggttacgctgacagggccagcgaaagcatcattggtgctatagcgcggcagttcaagttttcccgggtatgcaaaccgaaatcctcacttgaagagacggaagttctgtttgtattcattgggtacgatcgcaaggcccgtacgcacaattcttacaagctttcatcaaccttgaccaacatttatacaggttccagactccacgaagccggatgtgcaccctcatatcatgtggtgcgaggggatattgccacggccaccgaaggagtgattataaatgctgctaacagcaaaggacaacctggcggaggggtgtgcggagcgctgtataagaaattcccggaaagcttcgatttacagccgatcgaagtaggaaaagcgcgactggtcaaaggtgcagctaaacatatcattcatgccgtaggaccaaacttcaacaaagtttcggaggttgaaggtgacaaacagttggcagaggcttatgagtccatcgctaagattgtcaacgataacaattacaagtcagtagcgattccactgttgtccaccggcatcttttccgggaacaaagatcgactaacccaatcattgaaccatttgctgacagctttagacaccactgatgcagatgtagccatatactgcagggacaagaaatgggaaatgactctcaaggaagcagtggctaggagagaagcagtggaggagatatgcatatccgacgactcttcagtgacagaacctgatgcagagctggtgagggtgcatccgaagagttctttggctggaaggaagggctacagcacaagcgatggcaaaactttctcatatttggaagggaccaagtttcaccaggcggccaaggatatagcagaaattaatgccatgtggcccgttgcaacggaggccaatgagcaggtatgcatgtatatcctcggagaaagcatgagcagtattaggtcgaaatgccccgtcgaagagtcggaagcctccacaccacctagcacgctgccttgcttgtgcatccatgccatgactccagaaagagtacagcgcctaaaagcctcacgtccagaacaaattactgtgtgctcatcctttccattgccgaagtatagaatcactggtgtgcagaagatccaatgctcccagcctatattgttctcaccgaaagtgcctgcgtatattcatccaaggaagtatctcgtggaaacaccaccggtagacgagactccggagccatcggcagagaaccaatccacagaggggacacctgaacaaccaccacttataaccgaggatgagaccaggactagaacgcctgagccgatcatcatcgaagaggaagaagaggatagcataagtttgctgtcagatggcccgacccaccaggtgctgcaagtcgaggcagacattcacgggccgccctctgtatctagctcatcctggtccattcctcatgcatccgactttgatgtggacagtttatccatacttgacaccctggagggagctagcgtgaccagcggggcaacgtcagccgagactaactcttacttcgcaaagagtatggagtttctggcgcgaccggtgcctgcgcctcgaacagtattcaggaaccctccacatcccgctccgcgcacaagaacaccgtcacttgcacccagcagggcctgctcgagaaccagcctagtttccaccccgccaggcgtgaatagggtgatcactagagaggagctcgaggcgcttaccccgtcacgcactcctagcaggtcggtctcgagaaccagcctggtctccaacccgccaggcgtaaatagggtgattacaagagaggagtttgaggcgttcgtagcacaacaacaatgacggtttgatgcgggtgcatacatcttttcctccgacaccggtcaagggcatttacaacaaaaatcagtaaggcaaacggtgctatccgaagtggtgttggagaggaccgaattggagatttcgtatgccccgcgcctcgaccaagaaaaagaagaattactacgcaagaaattacagttaaatcccacacctgctaacagaagcagataccagtccaggaaggtggagaacatgaaagccataacagctagacgtattctgcaaggcctagggcattatttgaaggcagaaggaaaagtggagtgctaccgaaccctgcatcctgttcctttgtattcatctagtgtgaaccgtgccttttcaagccccaaggtcgcagtggaagcctgtaacgccatgttgaaagagaactttccgactgtggcttcttactgtattattccagagtacgatgcctatttggacatggttgacggagcttcatgctgcttagacactgccagtttttgccctgcaaagctgcgcagctttccaaagaaacactcctatttggaacccacaatacgatcggcagtgccttcagcgatccagaacacgctccagaacgtcctggcagctgccacaaaaagaaattgcaatgtcacgcaaatgagagaattgcccgtattggattcggcggcctttaatgtggaatgcttcaagaaatatgcgtgtaataatgaatattgggaaacgtttaaagaaaaccccatcaggcttactgaagaaaacgtggtaaattacattaccaaattaaaaggaccaaaagctgctgctctttttgcgaagacacataatttgaatatgttgcaggacataccaatggacaggtttgtaatggacttaaagagagacgtgaaagtgactccaggaacaaaacatactgaagaacggcccaaggtacaggtgatccaggctgccgatccgctagcaacagcgtatctgtgcggaatccaccgagagctggttaggagattaaatgcggtcctgcttccgaacattcatacactgtttgatatgtcggctgaagactttgacgctattatagccgagcacttccagcctggggattgtgttctggaaactgacatcgcgtcgtttgataaaagtgaggacgacgccatggctctgaccgcgttaatgattctggaagacttaggtgtggacgcagagctgttgacgctgattgaggcggctttcggcgaaatttcatcaatacatttgcccactaaaactaaatttaaattcggagccatgatgaaatctggaatgttcctcacactgtttgtgaacacagtcattaacattgtaatcgcaagcagagtgttgagagaacggctaaccggatcaccatgtgcagcattcattggagatgacaatatcgtgaaaggagtcaaatcggacaaattaatggcagacaggtgcgccacctggttgaatatggaagtcaagattatagatgctgtggtgggcgagaaagcgccttatttctgtggagggtttattttgtgtgactccgtgaccggcacagcgtgccgtgtggcagaccccctaaaaaggctgtttaagcttggcaaacctctggcagcagacgatgaacatgatgatgacaggagaagggcattgcatgaagagtcaacacgctggaaccgagtgggtattctttcagagctgtgcaaggcagtagaatcaaggtatgaaaccgtaggaacttccatcatagttatggccatgactactctagctagcagtgttaaatcattcagctacctgagaggggcccctataactctctacggctaacctgaatggactacgacatagtctagtccgccaagtctagcatatgatgggcacaagactgcacttctggtggtgcggcatcttcgccgtgctgaagtacctcgtgtgcacaagcagcgccgacgacggcagcattacagcccccgagcaaggcacaatggtgggcggcgtgattgccgagcctagcgctcagatgagcaccgccgccgacatggccaccggcaagagcgtggacagcgagtgggaggccttcttcagcttccacacaagcgtgaactggagcacaagcgaaacccaaggcaagatcctgttcaagcagagcctgggccccctgctgaacccctacctggagcacctggccaagctgtacgtggcctggagcggcagcatcgaggtgagattcagcattagcggcagcggggtgttcggcggcaaactcgccgccatcgtggtgcctcctggcgtggaccccgtgcagagcacaagcatgctgcagtacccccacgtgctgttcgacgctagacaagtggagcccgtgatcttcagcatccccgacctgagaagcaccctgtaccacctgatgagcgacacagacaccacaagcctggtgatcatggtgtacaacgacctgatcaacccctacgccaacgacgccaacagcagcggctgcatcgtgaccgtggaaaccaagcccggccccgacttcaagttccacctgctgaagccccccggcagcatgctgacccacggcagcgtgcctagcgacctgatccccaagacaagcagcctgtggatcggcaacagatactggagcgacatcaccgacttcgtgatcagacccttcgtgttccaagccaacagacacttcgacttcaaccaagaaaccgccggctggagcacccctagattcagacccatcagcgtgaccatcagcgagcagaacggcgccaagctgggcatcggcgtggccaccgactacatcgtccccgggatccctgacggctggcccgacaccaccatccccggcgaactgatccccgccggcgactacgccatcaccaacggcaccggcaacgacattaccaccgctaccggctacgacaccgccgacatcatcaagaacaacaccaacttcagaggcatgtacatctgcggcagcctgcagagagcctggggcgacaagaagatcagcaacaccgccttcatcaccacagccaccctggacggcgacaacaataacaagatcaacccctgcaacaccatcgatcagagcaagatcgtggtgttccaagacaaccacgtgggcaagaaggtgcagatcagcgacgacaccctggccctgctgggctacaccggcatcggcgagcaagccatcggcagcgacagagacagagtggtgagaatcagcaccctgcccgaaaccggcgctagaggcggcaaccaccccatcttctacaagaacagcatcaagctgggctacgtgatcagaagcatcgacgtgttcaacagccaaatcctgcacacaagcagacagctgagcctgaaccactacctgctgcccctggacagcttcgccgtgtacagaatcatcgacagcggcggcagctggttcgacatcggcatcgattccgacggcttcagcttcgtgggcgtgagcggcttcggcaagctggagttccccctgagcgctagctacatgggcattcagctggccaagatcagactggctagcaacatcagaagccccatgaccaagctggcttaagaattggcaagctgcttacatagaactcgcggcgattggcatgccgccttaaaatttttattttattttttcttttcttttccgaatcggattttgtttttaatatttcaaaaaaaaaaaaaaaaaaaaaaaaaa

SEQ ID NO: 12 - RNA, 9528 nt, synthetic construct
  source 1..9528: mol_type = other RNA
atgggcggcgcatgagagaagcccagaccaattacctacccaaaatggagaaagttcacgttgacatcgaggaagacagcccattcctcagagctttgcagcggagcttcccgcagtttgaggtagaagccaagcaggtcactgataatgaccatgctaatgccagagcgttttcgcatctggcttcaaaactgatcgaaacggaggtggacccatccgacacgatccttgacattggaagtgcgcccgcccgcagaatgtattctaagcacaagtatcattgtatctgtccgatgagatgtgcggaagatccggacagattgtataagtatgcaactaagctgaagaaaaactgtaaggaaataactgataaggaattggacaagaaaatgaaggagctggccgccgtcatgagcgaccctgacctggaaactgagactatgtgcctccacgacgacgagtcgtgtcgctacgaagggcaagtcgctgtttaccaggatgtatacgcggttgacggaccgacaagtctctatcaccaagccaataagggagttagagtcgcctactggataggctttgacaccaccccttttatgtttaagaacttggctggagcatatccatcatactctaccaactgggccgacgaaaccgtgttaacggctcgtaacataggcctatgcagctctgacgttatggagcggtcacgtagagggatgtccattcttagaaagaagtatttgaaaccatccaacaatgttctattctctgttggctcgaccatctaccacgagaagagggacttactgaggagctggcacctgccgtctgtatttcacttacgtggcaagcaaaattacacatgtcggtgtgagactatagttagttgcgacgggtacgtcgttaaaagaatagctatcagtccaggcctgtatgggaagccttcaggctatgctgctacgatgcaccgcgagggattcttgtgctgcaaagtgacagacacattgaacggggagagggtctcttttcccgtgtgcacgtatgtgccagctacattgtgtgaccaaatgactggcatactggcaacagatgtcagtgcggacgacgcgcaaaaactgctggttgggctcaaccagcgtatagtcgtcaacggtcgcacccagagaaacaccaataccatgaaaaattaccttttgcccgtagtggcccaggcatttgctaggtgggcaaaggaatataaggaagatcaagaagatgaaaggccactaggactacgagatagacagttagtcatggggtgttgttgggcttttagaaggcacaagataacatctatttataagcgcccggatacccaaaccatcatcaaagtgaacagcgatttccactcattcgtgctgcccaggataggcagtaacacattggagatcgggctgagaacaagaatcaggaaaatgttagaggagcacaaggagccgtcacctctcattaccgccgaggacgtacaagaagctaagtgcgcagccgatgaggctaaggaggtgcgtgaagccgaggagttgcgcgcagctctaccacctttggcagctgatgttgaggagcccactctggaggcagacgtcgacttgatgttacaagaggctggggccggctcagtggagacacctcgtggcttgataaaggttaccagctacgatggcgaggacaagatcggctcttacgctgtgctttctccgcaggctgtactcaagagtgaaaaattatcttgcatccaccctctcgctgaacaagtcatagtgataacacactctggccgaaaagggcgttatgccgtggaaccataccatggtaaagtagtggtgccagagggacatgcaatacccgtccaggactttcaagctctgagtgaaagtgccaccattgtgtacaacgaacgtgagttcgtaaacaggtacctgcaccatattgccacacatggaggagcgctgaacactgatgaagaatattacaaaactgtcaagcccagcgagcacgacggcgaatacctgtacgacatcgacaggaaacagtgcgtcaagaaagaactagtcactgggctagggctcacaggcgagctggtggatcctcccttccatgaattcgcctacgagagtctgagaacacgaccagccgctccttaccaagtaccaaccataggggtgtatggcgtgccaggatcaggcaagtctggcatcattaaaagcgcagtcaccaaaaaagatctagtggtgagcgccaagaaagaaaactgtgcagaaattataagggacgtcaagaaaatgaaagggctggacgtcaatgccagaactgtggactcagtgctcttgaatggatgcaaacaccccgtagagaccctgtatattgacgaagcttttgcttgtcatgcaggtactctcagagcgctcatagccattataagacctaaaaaggcagtgctctgcggggatcccaaacagtgcggtttttttaacatgatgtgcctgaaagtgcattttaaccacgagatttgcacacaagtcttccacaaaagcatctctcgccgttgcactaaatctgtgacttcggtcgtctcaaccttgttttacgacaaaaaaatgagaacgacgaatccgaaagagactaagattgtgattgacactaccggcagtaccaaacctaagcaggacgatctcattctcacttgtttcagagggtgggtgaagcagttgcaaatagattacaaaggcaacgaaataatgacggcagctgcctctcaagggctgacccgtaaaggtgtgtatgccgttcggtacaaggtgaatgaaaatcctctgtacgcacccacctcagaacatgtgaacgtcctactgacccgcacggaggaccgcatcgtgtggaaaacactagccggcgacccatggataaaaacactgactgccaagtaccctgggaatttcactgccacgatagaggagtggcaagcagagcatgatgccatcatgaggcacatcttggagagaccggaccctaccgacgtcttccagaataaggcaaacgtgtgttgggccaaggctttagtgccggtgctgaagaccgctggcatagacatgaccactgaacaatggaacactgtggattattttgaaacggacaaagctcactcagcagagatagtattgaaccaactatgcgtgaggttctttggactcgatctggactccggtctattttctgcacccactgttccgttatccattaggaataatcactgggataactccccgtcgcctaacatgtacgggctgaataaagaagtggtccgtcagctctctcgcaggtacccacaactgcctcgggcagttgccactggaagagtctatgacatgaacactggtacactgcgcaattatgatccgcgcataaacctagtacctgtaaacagaagactgcctcatgctttagtcctccaccataatgaacacccacagagtgacttttcttcattcgtcagcaaattgaagggcagaactgtcctggtggtcggggaaaagttgtccgtcccaggcaaaatggttgactggttgtcagaccggcctgaggctaccttcagagctcggctggatttaggcatcccaggtgatgtgcccaaatatgacataatatttgttaatgtgaggaccccatataaataccatcactatcagcagtgtgaagaccatgccattaagcttagcatgttgaccaagaaagcttgtctgcatctgaatcccggcggaacctgtgtcagcataggttatggttacgctgacagggccagcgaaagcatcattggtgctatagcgcggcagttcaagttttcccgggtatgcaaaccgaaatcctcacttgaagagacggaagttctgtttgtattcattgggtacgatcgcaaggcccgtacgcacaattcttacaagctttcatcaaccttgaccaacatttatacaggttccagactccacgaagccggatgtgcaccctcatatcatgtggtgcgaggggatattgccacggccaccgaaggagtgattataaatgctgctaacagcaaaggacaacctggcggaggggtgtgcggagcgctgtataagaaattcccggaaagcttcgatttacagccgatcgaagtaggaaaagcgcgactggtcaaaggtgcagctaaacatatcattcatgccgtaggaccaaacttcaacaaagtttcggaggttgaaggtgacaaacagttggcagaggcttatgagtccatcgctaagattgtcaacgataacaattacaagtcagtagcgattccactgttgtccaccggcatcttttccgggaacaaagatcgactaacccaatcattgaaccatttgctgacagctttagacaccactgatgcagatgtagccatatactgcagggacaagaaatgggaaatgactctcaaggaagcagtggctaggagagaagcagtggaggagatatgcatatccgacgactcttcagtgacagaacctgatgcagagctggtgagggtgcatccgaagagttctttggctggaaggaagggctacagcacaagcgatggcaaaactttctcatatttggaagggaccaagtttcaccaggcggccaaggatatagcagaaattaatgccatgtggcccgttgcaacggaggccaatgagcaggtatgcatgtatatcctcggagaaagcatgagcagtattaggtcgaaatgccccgtcgaagagtcggaagcctccacaccacctagcacgctgccttgcttgtgcatccatgccatgactccagaaagagtacagcgcctaaaagcctcacgtccagaacaaattactgtgtgctcatcctttccattgccgaagtatagaatcactggtgtgcagaagatccaatgctcccagcctatattgttctcaccgaaagtgcctgcgtatattcatccaaggaagtatctcgtggaaacaccaccggtagacgagactccggagccatcggcagagaaccaatccacagaggggacacctgaacaaccaccacttataaccgaggatgagaccaggactagaacgcctgagccgatcatcatcgaagaggaagaagaggatagcataagtttgctgtcagatggcccgacccaccaggtgctgcaagtcgaggcagacattcacgggccgccctctgtatctagctcatcctggtccattcctcatgcatccgactttgatgtggacagtttatccatacttgacaccctggagggagctagcgtgaccagcggggcaacgtcagccgagactaactcttacttcgcaaagagtatggagtttctggcgcgaccggtgcctgcgcctcgaacagtattcaggaaccctccacatcccgctccgcgcacaagaacaccgtcacttgcacccagcagggcctgctcgagaaccagcctagtttccaccccgccaggcgtgaatagggtgatcactagagaggagctcgaggcgcttaccccgtcacgcactcctagcaggtcggtctcgagaaccagcctggtctccaacccgccaggcgtaaatagggtgattacaagagaggagtttgaggcgttcgtagcacaacaacaatgacggtttgatgcgggtgcatacatcttttcctccgacaccggtcaagggcatttacaacaaaaatcagtaaggcaaacggtgctatccgaagtggtgttggagaggaccgaattggagatttcgtatgccccgcgcctcgaccaagaaaaagaagaattactacgcaagaaattacagttaaatcccacacctgctaacagaagcagataccagtccaggaaggtggagaacatgaaagccataacagctagacgtattctgcaaggcctagggcattatttgaaggcagaaggaaaagtggagtgctaccgaaccctgcatcctgttcctttgtattcatctagtgtgaaccgtgccttttcaagccccaaggtcgcagtggaagcctgtaacgccatgttgaaagagaactttccgactgtggcttcttactgtattattccagagtacgatgcctatttggacatggttgacggagcttcatgctgcttagacactgccagtttttgccctgcaaagctgcgcagctttccaaagaaacactcctatttggaacccacaatacgatcggcagtgccttcagcgatccagaacacgctccagaacgtcctggcagctgccacaaaaagaaattgcaatgtcacgcaaatgagagaattgcccgtattggattcggcggcctttaatgtggaatgcttcaagaaatatgcgtgtaataatgaatattgggaaacgtttaaagaaaaccccatcaggcttactgaagaaaacgtggtaaattacattaccaaattaaaaggaccaaaagctgctgctctttttgcgaagacacataatttgaatatgttgcaggacataccaatggacaggtttgtaatggacttaaagagagacgtgaaagtgactccaggaacaaaacatactgaagaacggcccaaggtacaggtgatccaggctgccgatccgctagcaacagcgtatctgtgcggaatccaccgagagctggttaggagattaaatgcggtcctgcttccgaacattcatacactgtttgatatgtcggctgaagactttgacgctattatagccgagcacttccagcctggggattgtgttctggaaactgacatcgcgtcgtttgataaaagtgaggacgacgccatggctctgaccgcgttaatgattctggaagacttaggtgtggacgcagagctgttgacgctgattgaggcggctttcggcgaaatttcatcaatacatttgcccactaaaactaaatttaaattcggagccatgatgaaatctggaatgttcctcacactgtttgtgaacacagtcattaacattgtaatcgcaagcagagtgttgagagaacggctaaccggatcaccatgtgcagcattcattggagatgacaatatcgtgaaaggagtcaaatcggacaaattaatggcagacaggtgcgccacctggttgaatatggaagtcaagattatagatgctgtggtgggcgagaaagcgccttatttctgtggagggtttattttgtgtgactccgtgaccggcacagcgtgccgtgtggcagaccccctaaaaaggctgtttaagcttggcaaacctctggcagcagacgatgaacatgatgatgacaggagaagggcattgcatgaagagtcaacacgctggaaccgagtgggtattctttcagagctgtgcaaggcagtagaatcaaggtatgaaaccgtaggaacttccatcatagttatggccatgactactctagctagcagtgttaaatcattcagctacctgagaggggcccctataactctctacggctaacctgaatggactacgacatagtctagtccgccaagtctagcatatgatgacaagactgcacttctggtggtgcggcatcttcgccgtgctgaagtatctggtctgcacaagcagcagcgacggcgccgtgcagcccgacggcgggcagcctgccgtgagaaacgagcgggctaccggcagcgggaacgggtccggcgggggcggcggggggggcagcggcggcgtgggcatcagcaccggcacatttaacaatcagaccgagttcaagttcctggagaacggctgggtggagatcaccgccaacagcagcagactggtgcacctgaacatgcccgagagcgagaactacaagagagtggtcgtgaacaacatggacaagaccgccgtgaagggcaacatggccctggacgacacccacgtgcagatcgtgaccccctggagcctggtggacgccaacgcctggggcgtgtggttcaaccccggcgactggcagctgatcgtgaacaccatgagcgagctgcacctggtgagcttcgagcaagagatcttcaacgtggtgctgaagaccgtgagcgagagcgccacacagccccccaccaaggtgtacaacaacgacctgaccgctagcctgatggtggccctggacagcaacaacaccatgcccttcacccccgccgccatgagaagcgaaaccctgggcttctacccctggaagcccaccatccccaccccctggagatactactttcagtgggacagaaccctgatccctagccacaccggcacaagcggcacccccaccaacgtgtactacggcaccgaccccgacgacgtgcagttctacaccatcgagaacagcgtgcccgtgcacctgctgagaaccggcgacgagttcgccaccggcaccttttttttcgactgcaagccctgcagactgacccacacctggcagaccaacagagccctgggcctgccccccttcctgaacagcctgcctcagagcgagggcgccaccaacttcggcgacatcggcgtgcagcaagacaagagaagaggcgtgacacagatgggcaacaccgactacatcaccgaggccaccatcatgcggcccgccgaggtgggctacagcgccccctactacagcttcgaggctagcacccaaggccccttcaagacacccatcgccgccggcagaggcggggctcagaccgacgagaaccaagccgccgacggcgaccctagatacgccttcggcagacagcacgggcagaagaccacaaccaccggcgaaacccccgagagactgacctacatcgcccaccaagacaccggcagataccccgagggcgactggattcagaacatcaacttcaacctgcccgtgaccaacgacaacgtgctgctgcccaccgaccccatcggcggcaagaccggcatcaactacaccaacatcttcaacacctacggccccctgaccgccctgaacaacgtgccccccgtgtaccccaacgggcagatctgggacaaggagttcgacaccgacctgaagcctagactgcacgtgaacgcccccttcgtgtgtcagaacaactgccccgggcagctgttcgtgaaggtggcccccaacctgaccaacgagtacgaccccgacgctagcgccaacatgagcagaatcgtgacctacagcgacttctggtggaagggcaagctggtgttcaaggccaagctgagagctagccacacctggaaccccattcagcagatgagcatcaacgtggacaatcagttcaactacgtgcccaacaacatcggcgccatgaagatcgtgtacgagaagagccaactggcccctagaaagctgtactaggaattggcaagctgcttacatagaactcgcggcgattggcatgccgccttaaaatttttattttattttttcttttcttttccgaatcggattttgtttttaatatttcaaaaaaaaaaaaaaaaaaaaaaaaaa

SEQ ID NO: 13 - protein, 15 aa, synthetic construct
TPPKPTTDPTDMSDC

SEQ ID NO: 14 - protein, 15 aa, synthetic construct
GKRRRGSRWQGHSGC

SEQ ID NO: 15 - protein, 15 aa, synthetic construct
KRSNDSRGESSGPNC

SEQ ID NO: 16 - protein, 18 aa, synthetic construct
CDDDVPTAPPKGMNNQSV

SEQ ID NO: 17 - protein, 15 aa, synthetic construct
STLPETGARGGNHPC

SEQ ID NO: 18 - protein, 15 aa, synthetic construct
TATLDGDNNNKINPC

SEQ ID NO: 19 - protein, 15 aa, synthetic construct
CQPDGGQPAVRNERA

SEQ ID NO: 20 - protein, 15 aa, synthetic construct
QTDENQAADGDPRYC